European Patent Specification EP 3 876 966 B1, published July 22, 2026. Title: METHODS AND COMPOSITIONS FOR TREATING OR PREVENTING THE DEVELOPMENT OF FOOD ALLERGIES. Applicant: Children's Medical Center Corporation. The sequence listing filed with the application follows.

SEQUENCE LISTING (6 sequences)

SEQ ID NO: 1 - DNA, 26381 bp, Homo sapiens
ccaacagatgaggagcacgtagaagcatcagggggtcagggagtcctggcaagagcagcaagggttaggggcaggggccgagcaggcagaggcctcagggaactgaacagtcactgggaggagtctgactgcatcctagagaagagacacagtcccccaaacctgccctctccatctcccctatgcctgtcacctgtcttaggtagaaatcacaggattctaaagtcacaaagacttgggtccaaatcatagctcacccatttattgttcttgtgtgagtccttgggcaaaatcattaatatctctgagaatccctccactcactgatcaatctggaataataatgtttccctgtggtgggtgctgtgaatatttacacaaagtaaaagcatggatttacataaagtgtcctgcaaagggcccagcacacagtaagtgattaataaatgctagttcccttcctttctcctgtcctgtttctcctcaaggctccatgcactggtccactggtctctcctcatgtcccctcctggtgccaggacactctgccagccactccttttccctgcctgctggagggccaggtgctcccgccttccaccctccgccctcctccctcccctgggccctgctccctgccctcctgggcagccagggcagccaggacggcaccaagggagctgccccatggacagggccccacagagacagcaccgagcctcacggggtaagaggcccatggccctgcctgcaggtggaagagactgctggaggttcagaggagggcagaaatggcaagagactgggcaagaagtgaggaggggagggagggacaagagtgcagaggagaaagccctgggttggcagggagtgaaactggaggagaaacaggaggaggggctggggagatgacagaggagaagaaatcgcaaaaggagagaaacaggaaagaaagggagaagcgggagaaggaagaaacaggttggagggtagatggggagggaagagccaagtcaggggagccagatctagacccagcgaggggtcagaatgtggacaggccctcccaggtgtgggcttaccccccaggaggcacagggacactgcttccttgatctggccaggaccccagacagcagtggccgggaggctggctgctccaccttctgttcattcaccagtggagaaacctgtcctttaaggagtgacagacttggggagtgtggcagggggaaccacaccctgtcagctgcccatgaccacgtagcctggtcctttcctcgccactcacccagggatgtgggatttcatctctgcagagaatgtggggcactgggccatcagcagggaaggacagaatgtcaggccgtccttggccccacccatggtccaagtcaggaaccccctcagagcaggatcgcagggccacaggcttggtcagctgtgagcatggaggaggaaagtttgagggccagagccaccaagctccagggccacctggtggaggaagaactggctgcctgggtgagcaaggggagcacccccaccacaggactgctctgaggtgcaaggctagaggccaggagccggtgccacgtcagggaggaagctgggtggggccaggcaggagcaaggggaggtgggcggggctgggtggggccttgccacctcggggcagtcttttctcctccctcaccccagcagagcccaggccatcaggccactcgcctccacacagcctagtgaccacggcctgccagtggggagcatctcccgggcagaagggcactgtgtgtgtgtgtgtgtgtgtgtgtgtgtgtgtgtgtgtgtatgtcaggtgtcaagactgaacagcagaaggaaaaaaataacagaatagagtcagaggttagggaagctatagggggtatagggcatggttgaagggctttctgagacaaaagactggccatgtgttctgtgatgagctgctatgtggatgtaggaaatgggccaaggtctggcaggggaatcctctttccaggggctccctggctaggtgtttcatagatgttaactgcatgaatgggtgacacccccccacccaccaaccatgctccagctaaggccctcccctcaacggctgctccccctggaggtccgagtatccatgtgacccccatcgacccactcatgctccctactgcccaatctccacccagacccggccacgcagcagcagcagagaagggaggccttcctcttcaggctggtaggccagggaagcctggcccgtggaagccagagaggggtctgtatttgcaactctcccctcctcttcctccaaacatcctctccccctactcccaacccccacatctctgaagccctggtgttttcaggcatagataagcaaccaagagatttcagtcccacagagatttaactctggctgtaggatatttcttgtgcacctccaatgaaattacaaagtaaataagaccaacacagtccctgccttcacagggctttacaatttggcaggaaagacccatttcatagacaatgacacaattacagcagttaggtgacagttggtgacatggtgagtgccaggaaataaaatgcaaggagctaaatgtgtcagcacaagggcaggggaagggggtgtgtgtggcttctccaaggaagaaacataatcagagacctgagggagaaagagaagttggctagattaaggggtacaggagggacaggcattctaggcaaaggagcagcttgggggagtcccagaggcagtgaggagcctgacacttctgggtacctggaagagggccagtgtggcccaagggcagaggaggagagaggggcactgcagggggtggcctgcctgcccttcagacgccaggctctgagggaaggagtgcggcagtgggatcctaggagtggggaaagtgtctcagcccctcatgatcttcaacctttgacgtcaaccccctctcttgtctttacagagctgctggctgcaaagaagacccacacctgtgagtagggggtccggggcaagaaaatggctggggcataatgagatggagaataattcagcaagtgatctgtggggggactgaggttggacagaggtggaggagtcaggaagagatggcaggcaacaggaaagcaaggggaggtgcgaggaaaccacagatcagggcagtgggaggagatgaggaagaagcctgaagcatgaaaggaaacactgtaaagaaaccaggagagaacaaaggaaaagggaaccgccttgtgaaaaaaggcgaggagaaatgctggacagaggcagggagatgggagggggtggggccgactgccaggccggggaaggaaggagatagaggtaggggggtgtgcggaggcggggtggcctcaggaactcaggaactcagcgctgctgccaagggagacagggagcctgcaccaggctttttttttttttttttgagacagagtctcacactgtcgcctgggcgggagtacgatggcacaatctcggctcactgcaacctccacctcccaggttcaagcgattctcctgcctcagcctctcgagtagctgggactacaggcacccaccaccacgcctggctaatttttgtatttttagtagagacggggtttcaccatgttggtcaggctggtctcagactcttgaccttgtgatccacccctctcggcctcccaaagtgctgagattacaggcatgggccactgtgcccagcctgcaccaagctctgtggtcctgagccaggtttggtgttcatctctgtggttaacacatcctgaggtgtgaacaagcctggagccagcctgtgcaggactagagagcaggagagctttatctctgtaggaaacagaatggacaggggcactctgtgtcctggggccctgaaagccagactacagcaggtaagaagggcactagagctcagagaggacttcccagtggacgctagtgaataagaatcctctctagggaccactcagcacatcagctctcctctcctagtttgtggcaaaggctagtcccccagagaatgcacacagtcccaaagctatgcccatcagggccatgcgtgcccttctgtgagcatgggtccctgaatcgagaggatccctccagggtaggagtggccacaccatttctccatagccgtcccttgactgccttgccagttcctcctgagagctcactgccatctcgcccaatgccaaaattgtctagagcctccctgttccaagtagagacatctcagagagcaaagcattgcccttctccatgagctgggcagcccagggctgagggccatccaggatgctacctcctcctgggtgggggttgctttgctcagcataatcctgatcagtgtctcgcctgcccctagccacagggccccacggaaatgctgagcagggccccgggaggaaagcgggtcagggagtgacgcgggtgagctgggggaggggggtcacggaccttatgtgggtggggggagtagggggactttcggagcagcaggaactgggagaggtcaaaccctattcctacccttaacccctgacctcagaaacctcagccaggactatacctccttatccctttcccatcccaccagtcctcgtgtccccaccccaagagtgttgtcctgaggatccaggctgacagcctctcccccactccacggcccagctcctgaagccccaggaaggcccaggaaggcaaggaaaggcctgtgcctggatgagagggtctggagtcccagcaagatcagacacctctcaggagtttgccccacagaatccaggagacattaaggcctcccccaggccgagagactctgaaaattggctcctgaattgagacaaccccaagatgggggtccaagatggggaacccgggggaactccccagaccaagagggagcctgaatactgaggggccctgaagagggactctcaaagccaatgtaccccacaaagcacctaagaggctgagaaggtctctggaattgtttggcccctgagaaggacccccctcccccaggccaaaaaacactccagagagactcacataccgagggacctcccaggctgagacaccctcaaaagcagacttgaaccagagaaaccctcccatccttcaagtgggatccgaagccagtctgcctgggcttgaatcctgactctgccacttactagctgtgtaaccttgggcaagttacttaacctctctgtgtctcactttcctcctcgaaatgaggataatggtagctacttcataaagtttttttattttttctttttgagacagagtcttactcagttgctcaggctgtagtgcagtggcattatctcagctcactgcaaactccgcctcccgggttcaagcgattctcctgcctcagccccctgagtagctgggactacaggtgctcgccaccatgcctggctaatttttgtatttttagtagagatggggtttcaccatgttggccaggccggtctcgaactcctaacctcaggtgatccacccaccttgggctcccaaagtgctgggattacaggcgtgagccactgcccccggcccacataaagtattttgtgaggattagattatccacataaaacatcgagaaccatttctgacacataatagtaagcactattattatgattatgagtatgatgatggtgatgatgatcattatctacactccaatttcagcagtttggctcctaaggaaatttctggtttccttctgtggattgtgggtatttgcctggtgattattactgcttctatcatttccatgtattccctagcgcaagatatatgtggtgtctgcagggaggagcgtgggcatgggagtggtgggacagccccccaggctgcaccacactgggtatggctgttggcagtccacagggtgtcaggtggcacatgccaccaccccaggcagacatcctgtgacttacctctgaaaacatccctgtccctgaagtcacctggcaaagagggtcaggcttggaaggtcctcgggggtaggaggagtagaaatttggcttcaggctcgtgtgagctccattctggctccccagccagaactaccctggcgggtggaaacagcttttaccgcgtgtggctgtcgcatgtggttttggaattttccaacgccccctacgattggctgcccctcccctcacaccctgccccaggcccagattggccacgtggggcgcctgtcatcctactcactgcaccccttgggggtggggtggggggttgtcacttggccacctgtgtggtgcagagcttaaaccccccagtccagaagcactgggggagagagctaggtgcagagcttcaggctgaggcgctgctgagagggcctcgccccgcctctgccgccagctgcaccccactcctggaccaccccctgctgagaaggacagggagccaaggccggcagagccaaggctcagtcatgagaagtaagtgaatggggccacctgggggcgggggagcctggaccctgtcgtcacccctctggaaaggaggatgtcttgggaacagtgtgagcaaatctgagcaaagcagggtgcgtcctggtcaaggtcaagatctgttgggagatgggtggagcagctggggagtcctgctggccaggcggctccctgacagcagcaatggtaagaggactgttgaggaattcctgagttccaaaaagaacctccaaaagtatctgaggtatccaggcccttaattttacaaaaagactgagagccaaggaggccgcgtacttggcccaatgttacacagctggtatctgatgggggctggtaattactaggggccctgaacgcactctcctgttacagtgtttcccttgttacggtgtttccctctgtgcctccagcctgcttgtgagtaaaaggaggccagagcagttgctgtgctctgaagcaacaggacagcgagagtcaactgaggttggcaggcagcagggcacagaatccccgcgtccaggcctcaaagccaccaggctttctgcccaatccagggacatgaggactatgtggaatccagtcagggtgcacccgggcacatgcctgcgtgtgtgtgcatgtgtgtgtgtgcgtgtgtgtgtggggtgtgtgtgtatgtgtgtgtgtggttctccagggtcagtcacccatttgaccggggaagcaaggcaatggagatgggattggaaagacctcggcctcacccttttcctggcttggagccctgggccaacagttggtgggcagatgtctggggttcctgtgccttccagcagagcaagggtgggcaacctcaggaagtcccctgtatttgttgtgaagggaagccagggaagccagagaagctctcagagcacaaggtgaaggaggaaaagggaagccccatgcccctgtggctgaggcctgaagcagccccagcttcaacctggggtcttcccacaagccacagaagggaggccgtattgagtcctggaaagacccctggactgacagtgtaagaccaggcacttgtgccgcctatcactggctagccatatagacttagacaagccaagtcactgggccctggtctaccatccgcaaaacaagggagctgaattttaagatagaacaacaaaaccaactatggagagtctcccattccaaaggcccagggccaagagagagcccagtgccctaaggcaggcatccccaagggtgatgatggagactcagctctcccagaggttagaaggaagggaaaccaaggaaagaaaagaattccacttctgtgacagggactgaggccacagtgcaggcatatgagctggggtggataaggagggctggagagaagagccaacagcttctacacagaggaaagggccccttggagcttccgtttcccttctagcttctctctattagcagcaaacgctggcagactggtcttcccagagatggcccctaatgagcaaatcaaccctgggatgaaatgactaggtgtgcttctagcccagcagcggggcaggagtccccaggaggggctgagggagacacttggccagctctccattattcccacccccaccacacacacacagccccacccaggcggggaagtaggagagagggcctcctccaacgagggggtcagtgccactggtccttctcacttggacatttacaggtatctcatagccccaagttatctgaccccaatgagtgccaaccaccaccagcccctccaaccgccgatggcaaaagtcaaagcacatggggcttgggactgtgacacacccagagaccaagggcccgacaaaaggagcagaaacaaatcaagaaataaggagagatgcagaggcccaactcagagggcgagtttctggaacacctagggagagagtaatgtccagctggaggtgtggttggagaaacaccaatagagccaaacgcatggaggtgcagccgggcgtggtggctcatgcctataatcccacttcaggaggctgaggcttgaggccaggagtttgagaccagcctgggcaacaaagtgagccgctgtccctacaaaaaaagttttttttaattcgctgggcatggtggcgtgtacctgtagtcccagctactcaggagactgaggcaggaggatcgtttgagcccaggagttcaaggctgcagtgagctatgatcaatgtcacagcaccctagcttaggtgacagagcgagaccctgtctcttaaacaaacaaacaaacatgaaggtgtgaagcccagaaacagagctggaatgcagaagatcacaaggcacatagacacagggagaggcggagagaaaagataactggcagtaaagggaagacagggagacacagggtctaggcaagcggtaagagggaagtagggtggctctgacaaggatggcaccagcaccctgccatccgacctgctgctgtcaagtggagataatgtgtctgtacgccaaagagactcccagccagccagacggagggtagcccagacatcttcccctaagggcatggccagcgtggcgccaataggcactcaggccctggcatttggtctggatggggaggtgggaggccgaggggtgtgaggtcactgtctatgagctgatctttcttaggtttggtcatgatcatgaggaacagtgggccagaaaggactccaagtccccagggtacacagatatcaccctgagagcccagggccatcttaggactccgtgaagggcttcttccttcctttcatcactccagcacccttctctttccccgtcttcccattcctaacagaaataccaaaccaccgagcccaaggtgctagactctgaaaagactcagcttgtcccagcacaatgaaaatattcggtccctaccaagggctcctccccatcccctgccgctgtgctgctgactcaaactaacagggaacaggactttccaagggctaaggtctctcccaggcgggcagcccaaggcccgcgctcctgttcccatatagctagtcctttctgaagtctcacctccacgcctgctgctgcagtgcagccccttccctggggctctgaggctcaaaaaggatggagatgtctatttcgggggagggacagtaacaaggcagggcctcagggccagagccaaggtctttctgggtccactaccctcctggagcagtgaaggtgctctgggatgagggacagatggccctgaaggcagggaaggtgctgatggtgacgtctgggctcccactcgccagagcttcctcctagtgattcatcccctcccccattcactggttgttttcactcgcctttctccagtcccagactgtgggggtggcggaggcaccaggagggggtttcgggtggctggctggctgtcattcatggcttttcaaaaccccagactctccctcgcccacctgagttttagcttcactattttctcagccccaggatctgggtgtttcagcagaaaattctcaccaggagctgcggtgagggccctggcctgggctgggggtagtgttcgccaggtagaaccacttctcccccagcccccacccagccctcccgctcctgctcccctgtggtggcacccaccaccttggtttccagctttgcagaagctgggggaactgagagctgagaaaggagggaggctggtgacaggttggggtgtgcaagtgacccctgaccggagctgtggtctcggtggggatcgagacagagagttctggctgtggggagaggaggagctcaagctaaggaaagagatgcattcctctttctcactcattcattcattctgcaaagggaggcataccaagatgtatggaaacctagtctataccctaaaggggctgtggtgttcctgaggagtccccgggaaccctgttgttgatatataagtcatcccacttggccttagagaaaggggtaagggcaggaggaggctgggacctcagaggaagagttgggacagagggaataatatctcttgggatctttatacaaacaggagtcctggctttagttctgtgggtttcctctgtgaattctgttcctagaccaccacaatcacctcacacttttacccctacagccaaataaccatgtcctctacccaggtctccggtgtgcatttgggcgtcttatcctcataaagtatatagcttaaggcttgagggcactggctgcagaattacagagatctaggttcaaatgccagatctgccacttctggctgtgtgaccttagtcaagctgtttattctctctaggcctcagttttctcatctgtaagatgaggatgatactagcagggcctatttcacagggtggttgtgatcattgaatgaaaatgcatgtaaagcctggcacagagtaagaattcagccaatgcttatgtctatcattatcctttctccttaatcagtatccactggagaaaaaggagagagaaagaggagaggaaaaggcccagctctagattgacgaggcaccaggaggagatgaggaccccggggtttctctgtgtgaacccattctctaccatgatggtgggggggtggtggttctggggtttgagaggagagatccccctgggttgcagcccctcccctgctcctaccacttcctctctgtggcatagggcacctggacagggcccagggttggcttcctaagctggcacagggccaggctctggaagtactcaaagcactatcattgaatctcacagctgtgagaggctcgattagaggaggatggaggactttgcctctaccgtatttcccctcataggaggagctactaggatgctcctgggggtacttcagtctctaaagcaattcagaggagattcagtttctttttctagtattgtctcagaatgaagtcttagaggtcacactggatggcagaaaagatgcaagaatgagctcaggaaaagatcgccaaccccagccccactccctggaaggagcagcctggcaaaaaggcaggaatagggactaagttcttgctactcaaagtataagctgaagaccagtaagcttaggcaccaactaagagctgaccaaagtgcagaatcttgagtcccacctcagatccccaggtaatcttgtttgagatgcagaaagccatagtcattcagtcattagatgacttaaggagctggcgggtgcatttgggcatttgtctctccttttggaagatgtggaattggagttttcttttggagaaagctctctctcaggagagagctacagtgagagagctgcaggtgagatgcaaagatctttccaagacagcaggcgagggtagagttagggctgccatgggagcagtggtgcaggggctggttcgaggttcctgacctttgcttggctctagttcctggcactggcaggcccttagatggtaagttcctggcaggcctggctccagggcaacagtttgagtaatcctgtgattactcagctccttctccccaatctgagttcccaccacctgctgcttcagggacgtgtctcccaggggtagcttttgaaggtgagttatcatcagaggtgttttcagctcctctcaccaacccccaagtctaccagcccccttcccgttctcccccaccccttctctacaagtaacacacaccctcatgtacacagcactggtactttctttctgaggtttgggtggatggcattgaagggagtgcaggtggcaggggaaggaggggggagcaggactagagggcctgaagtgctgagggggccatgggttgggcaaaggccaggatacaagcgtggattttctgtgtttcagtgtttccgcagccgtctctccatccctagatctatgtctctgtttttcctggacccaaacctcttggtctctccagctcagtgaggctagggggtctgacattctagctcagagtctttggccttgtgtgtctgtctcactgggtacttctgtcttggactgggaggatggaggatgggctgaccaggtggctggagtccaaggctttggtgtcgcccaaacatgggtatttgcgaagggggtccttgactggccgcatcttcctatgagaaggtcaaggtcttggtgacactgttgtgaggttcctagggccaggagaagcagtgggtcaagcatggggcagggagatgtgtctggggtcaccatgtggtcagcacacacacgcacgcggatgtggctcttggagaagggaagaggcagggaggcctgtggttgactgctgggccagagcccgagttcccactgcggcttggcctaatctccctcccgcttacttttttgggtggcccacgttggtttctcccatctctggtcttaggccactgaaaagagagatgccacagtgttggagggggaggtgttgggcaagaacagagtccacagggcccgagtgctcctctcagccttgccaggcccactggtcttctcagcctgacctctgctcaggagtaacttgaatacacagtgctttccattggtgatatcatttcattactctctgttacctacaatcaccccatggacaggcaataatacttttatcctgatcttgctgacaagaaaacgtaggtctagagggagaatctaagtgactagaagtatgggggccccaacgttttctgcccctgttccagacacccagtgccctcttattctctcttcccctccatgtattaaaatctgctcttaatttactggaaagaacctggaaaactcacttaccgcctggtcctggggggaccacagcttacagtgtgagcactggaagcttgctgctgggcaggcacgtgtggctgggggttgggtgaggaattgagtgctaatgaagggatttcagatacccatgtgccctgtccccgtcagggtcagctactgcctctgactcacctcaagtctggcctgagggatgatggtttaagaatgatggaaataatattttggggaatggcgggcaagccatggtctccctgcccacttcacatcaacaggccctacatgtgaccagtgtccaggccagggactggaggtgagatcacagcaatgtgcattcgccctccagagaggctgccacttcttttgcccctttggtgggagacacgtcatagattaaaaggggctttggcccttctcttcacttttctggcctgtcccgccccagggctccccactcagaggggaggcagcaggtcagtgatggtggaaaagagacccatgtgctctgggaaatgctaaaaacacctacagtaaccagggatcccaagctttgcccagctacctttcaaggaagagctgggagaaggcctcctgtggtcccatgaagctcagcagagagtcgtgggcattgacaggaacagggcaaagcagagatgagcttagggccagcagcaaaccacaggggtagggaagcaggtacaggttacagtgagttcagtgggagagagaacccggggtcctagtgccccatgagcagacactaacatacaaatatgcacgtgtggacgcaggagcaaccagatatgtcgtaggctcacaaatgacacatacttttcttgcatatgcacacccacaagcacaccttcaaacatgcccactgaaatgtgtacccgaaaagacaggtacacagaacagcataatggaaagctcaggggaactgggatgtagatccagctctcaggcaaactagcctatgaccctggcccaaccgctttgcctcatctggcttagtccttcatcggtaaatgaagaggttgaatgagatggtctctagtctcagccatttttaacattgatgattcatgttcacacaaatggatacagatgcctttgtacaaacataagtgttcacactcagacacacggatgtacacaaagccaccctctctctgctctggggccaagagcctaagagccctggctaattctttccctaggctctcaggcatccagcagagctggggtgttgagcccccgtttcctgggttcctccctgccaccccctcaccctgtctctgtatagcacctccctgagccttcactgtctggctgggaaggactggcatctctgcctatcccccaccccttgtgtaccacatcttcctgctataccctacactttgcccatgggagctgagccccagcgagggagggaggcacagaggaagccccttcggcgggaagcaggtgttgtgaggccgtgaggagtcctatgtcccaaggcgggagggaggcaactggagcttttcaactcgaagggctgagcaggtggcccctctgcagctgctttctctgcctccatagcactgatacaactcccggccacccctccacactcccctcctctgtgaaacaaacacagcttcctcacaccctttgctgagaagcatttggcatttcacttccccttccattttgcaagagggaaacagcaagctggagctggttggagaagtagtggaagcaccaggtacctgtatctgcagcccaggtacatggtggttgaatgcagaaaagcctcctgggctgacctacttctctttctctcttccagcacaaattgaagtgatcccttgcaaaatctgtggggacaagtcgtctgggatccactacggggttatcacctgtgaggggtgcaaggtgagtcataggcatgtgtatgcatgcatgtgtgcgtgtgcatacacaagcgcgcgcgcgcgcacacacacacacacacacagtgtctccttagagataaacaagggggttaatggcctttgttctgactccagggatgatctcctgggcagccaggaaaatgcctgagtagcgccttcctgcagggccctcaacactggcagggccctgtcttaagctggggaaatgactacaggataaattgcaattacacaaatagatggaggagagagaaaactgacaggtcgtgggatgtagaaaagctgccagagcttgtgggctggaggcctttgtgagtgagctgggcctgaccaggataagcagtcttgccctccacctgctttccccagggcttcttccgccggagccagcgctgtaacgcggcctactcctgcacccgtcagcagaactgccccatcgaccgcaccagccgaaaccgatgccagcactgccgcctgcagaaatgcctggcgctgggcatgtcccgagatggtgaggccaagtcgacagccccctggggttttcctggtgtctccagaggggcagcctggcctgctgagctagacaaggcttaacctgcaagacggcccatcctctggtctcctctccattcctccccgttacaaccccttgtctcctcccctccagggatggatgggtcacccccatcaaagttctttggagtccccaactttaggctttgctagaacaaacatcctctttccaaggtcccatacctcttcatctcttcttacttggaacgaattctcctcactctgctgccctctggcccagctcccatgcagctctggcaccttcccctgctaccctgttgttgtagttctagctctatctccttttctaatcccccattcccatacttggacacaggactatagccaggaatggaaacagaattggcctgagaacaaccagagggtggtcgtgggggagggctggtgttcctggtgccttatccaccctcctcacccaccacctcctcaccagtctccctgcacacctccaccaccacagaaggagcctagggtggagctgggggggcatgaggtgatgaggagccagaaggagcccgtcagcacttttcagtgcccaaaataacaaagcaaaaggaagcacgcaggggtgcaaaggggcaggcggggcgaggggctgtgcccctacacctgggaggggtggcggggggagtaaaaaggcaggaaagagagagcagaagaggatgttcagaaacaagccgcggagcccgggttgggctgtggtgagtatctaggtcaccagggagcctgcaggcctgaccacagggagacctgtgttctcagctctcctcttcctccgaccctcccaaagaggcgaggtgaccccaatacagcttgaggccctctgctcgaccacccccagccccaagatctggaggccagaatccccagcctagactcattgcttgaattctgccatgattcaaatctgatttagaacttagaagattttgcttagcagattgaaatggcagactggacagaccccagaagcaaacaagagtgagaggtggacggggtcttgagcataagttccctaaaggctagagaagctgtgcttggagtcagccattcagagagcagcaagttaatcctttaatgaccaaatgcctcctgaccctgccctgtgccatgttctcctgcctcataaacccctggtccctggacctctttcagctgtcaagttcggccgcatgtccaagaagcagagggacagcctgcatgcagaagtgcagaaacagctgcagcagcggcaacagcagcaacaggaaccagtggtcaagacccctccagcaggggcccaaggagcagataccctcacctacaccttggggctcccagacgggcagctgcccctgggctcctcgcctgacctgcctgaggcttctgcctgtccccctggcctcctgaaagcctcaggctctgggccctcatattccaacaacttggccaaggcagggctcaatggggcctcatgccaccttgaatacagccctgagcggggcaaggctgagggcagagagagcttctatagcacaggcagccagctgacccctgaccgatgtggacttcgttttgaggaacacaggcatcctgggcttggggaactgggacagggcccagacagctacggcagccccagtttccgcagcacaccggaggcaccctatgcctccctgacagagataggtgagcagctggggaggtggagagggtggtagagatgagggaggggtttccaccagtaccccgtatcaatcaaacatgcgcctgagggaattgaggggtccagacgaggggcggagggaggaggcggagcaggataggccaggctgagaagtgcccttgcatgggtaggcgtaggagctggctgagatcaagccatgccttccttctccggccccagagcacctggtgcagagcgtctgcaagtcctacagggagacatgccagctgcggctggaggacctgctgcggcagcgctccaacatcttctcccgggaggaagtgactggctaccagaggaaggtgaggccaggagacctgcaggaagggaacgtatcccacccccaccgggagagttcagagatggctacctgcgcacgactgggtcctggggcagggcgggacatcacagacacaggctggccaacaagcatgtgcacaccttttatgtacagttgcgaatgtgtgtatctgtctacaccccagcagatggatgagcgcttttccttagttcttgcctattaaaattgtacctggccttcatcctacctcctctaccatgcagaccttggtgcaccctccttcctcctcttccatcaacaataacaataatcagaaccctgattaccatttgttaaacaccccttctctgccaggcattgtgctaaacgctttatgtaaattatcctcagcccctaccacaaccaacctatgagggtggcatttattcctacttttaacagacagaaactgagcctagaggggttaataggtttcctcaaagtcacaaagtggtggaaccaaagtcaaattcagattcatcaggctccaaagtttatgctgccttttcgatcacactctcataccacctgctctaaacacactcgtttggcacttcacatttgcttctccaggttattgagaccttgggcataacctttgtgggggaaggggcagctgtatgtcctgttcacctcaacgagatataccttgttggagggcaaagctgtatctcatactttttggattccctcacaacagctaactcggtgtcagcagccggtaggtgctcagtgtgtgggactcactggcaggaatctgtgcatttgtgctaagaccaggcttttgaaaatgctagttgagaacataggagttcagagcctaccccttgcagtttattaggtggggctccagggctcaggaggatcacagggccacacagagcgctacagcgggaccctcctccctccctgcagtccatgtgggagatgtgggaacggtgtgcccaccacctcaccgaggccattcagtacgtggtggagttcgccaagaggctctcaggctttatggagctctgccagaatgaccagattgtgcttctcaaagcaggtgcccagggatgggtgggcaggcctggggacaaggggacagagccaagtggagggaggtggcttaaggaaatcagggggacagagtcagatcctggctttgcttgacactgtccctgcatcttctctccccactgcccaggagcaatggaagtggtgctggttaggatgtgccgggcctacaatgctgacaaccgcacggtcttttttgaaggcaaatacggtggcatggagctgttccgagccttgggtgaggggcagggagaaatgagagggaagattctgatgccaaccccaggcaaagctttgtgacccagggcaccctcttttcagggcgaattgccccctctgctctaaacacaataagggcggtgtcctcgggcaccatcgctccagccactctctcacttttctcatttccactccatcaggctgcagcgagctcatcagctccatctttgacttctcccactccctaagtgccttgcacttttccgaggatgagattgccctctacacagcccttgttctcatcaatgcccgtgagtgttgctgggcttgggtgaaggacattcaggtggcaggggcatggcagatattgaagaagagtctagaccttcagatgtagttaaatctgggaaattgctttaaatagcagaatgagccctactcagtattgctataaaataaaatgagttaaaataaagattcagaggactctcagagagggacaagagcagcataaggtggggttgtgggaagtggggagaaatgaggttgagaggaaatgagccactttcctgacagaaatgtgtctgattgttagtctatggcagtgatttcattgtagcacacatcagaatcacctggggagctttaaaaactattgctgcctgggtcccacttccagagattccagtgtacatgtgctccatgacttatgatggggttatgtcccaataaacctatcgtaagttgaaaatatggtaagttgaaattgcatttaacacgcctaacttactgaacaccatagcttagcctagcctaccttaaatgtgctcagaatgcttacattagcctacagtctggcaaaagcatataacacaaagcctattttataataaagtgttgaatagctcatgtaatttattgaatatggttctaaaagtgaacagcaggatggttgcatgggtattcaaagtatggtttctactgaatgcaagtggctttctcaccaacataaaatcaaaaaatagtaagtcaactcatcataagactgggaccatctgtaattgataaggggtgcactgaattttaacagccacccccaggccaccaagattaagaatcactgctctgtgtgaactaattttaaggctgtatgcctataataggaagactctggatatcctatccactcccctggcatggagtagctgggctgagccagatgaatactaaatattcagagaacctagggaagtgggtcaagctgctaacctgagtttgcagatcgagactatcagtcttctggctctgccagtgagtggacacctaaatatgcccttcaaactagaagataaaaactttaaagatgacttctggatattttatagaatcagggcaaaagttagtcacagattgctgcaagccccctggtgcaggcctgggcaccttcaggaaggccacctcctatcaggagcccttttcgtacatgggggagctcttttccaactcttgttacccctatgacagaatcctagtgcctagcattgaatgagctatgtggaatatcaggttaccagggagaaggtagcttggagtcaggagatcagaaattctcatacctttcatctcttcccagttttccttgtagacagctagccaagcccaacgtccagagcttaccattatcaaaccaaggcacacacatgcacgcgctcagcttagaagacctctatccagcacagatgtccacaaagatacacccttttgttgggagttaatgtccatgttctttcttgttctcattacggtcccaccccctcctccagatcggccagggctccaagagaaaaggaaagtagaacagctgcagtacaatctggagctggcctttcatcatcatctctgcaagactcatcgccaaagcatcctggcaaaggtaggagcagtccctggggtagaagaggccaggcccatcgctagctctgtaacatcagagtttgcgagggccggggtctgtgggtacagaggagggagtgcgggagtaccactctctgttagagagcttgcatcagcagtgggaactaagggaatgaacagctacttccacgtgcataaagactggaaagttagagggcctgggattgggagggacctccagggaacaattcagtttaatatagccagcacttacccagcacctgcttgtacaaggcactgtggaaagacacagagatttggtcgctgcccccaccaagagattttaatctggtatgaagaagagatctgtgtatcactaactctaacatagagtagaatgtggtatgtgatataataataatgcaattaacagagtgcttttgctgacatgctttctcatcctcatggcaacccagtcaataggacaggtgttcaaatctccctgtgtagcagccgggcacagtggctcacgcctgtaatcccaacactttgggaggccaaggcgggtggatcacctgaggtcaggagttcgagaccagcctgactaacatggtgaaaccccatctctactaaaaataaaaaaaattagccaggcatggtggcaggcgcctgtagacccagctacttgggaggctgaggcaggataatcgcttgaaaccgggaggcagatgttgcagtgagccaagattgtgccattgcactccagcctgggcaacaagagcaaactctgtctcaaaaaaaaaaaaaaaatctccttgtagctatcaggagacttcagtgacttaaatgcaagattgaatcccagtgctctttgcgctctttctatccctgtgtcccctatgtataactataataagtgacaccaggaaaatgttatgagagtataaaacagggattaaaaataatttgggggtaaaaggagtgggtcataaatacttcccagggaagatgacatttatactaggccatgaatgatgtaagattttaacaggcattcatgggggtggggcaggcattccaggcttagggaacaataggagcaaaacaaaaaaaatgaaaaaaaatccttttcctgaggtttaaccaaaaaaatggatgagatgagtatgagaggctggggataattgttttatgggatttgggtgtgggactagggtacaatgaagaccaagaacaacaggagaaaaataaggaggcaaaatagtgtgtatgtggagaatcactcatggtacatcctcactaaagtgtaaaatcaggagctgggatagactggtggggcagaagagcaccagatgatcagcctgaaaattaggtcaggggcaaatcagagaggactttcaatgccatataagcgttaaagctttatttctaggccacagggagctccaaaggctagaaaaatgacacaatcagagctgtcatttaggcaatttactttggaaccagtataaaggaaccatttatgtaattattcaagcaggcctttgctatgtgccaggcacagggctgggtgttaaggatacagcaatgacttacacggtctgtgctctcaagaacttgaactttaatctgctacaggatggatttgaaggaggagagacaggaatctgggagagcaattggaaagcacatccggttggatctgctttcaaaatacatcaccttccctactattaccaccaccctggcccctaccagctctcagctttcacttggactttaagagaggcctcctaactgagcccctgttccaccctcatctgccctgtagcaaccacacctactccgcacccacggtagcccttttaaaaatgcaatctcatcatgccctactcctgtggtttttttcttgtttttgttgttgttgtttgtttgttctgtttgtttgttttgaggcagacttgctctgtcgcccaggctggagtgcagtggtgtgatctcggctcactgcaacctccacctcccaggttcaagcgattgtcctgcctcagcctcctgagtagcttggattacagggattacacgcccggctaatttttgtatttttagtagagacagggtttcaccatgttggccaggctggtctcgaactcctgacctcaggtgatctgcccaccttggcctcccaaagtgttgggattacaggcgtgaaccaccacacctggccttgactcctgttctcagccctcctgtagctgcctgtgatgccgagaatcaaatctagagtctgcgtcatggtcaagtggctcataacatgatccctgccttcttttctcacttgatcttccactgccccttcaaacacccattgcagccacacttgcttccttgctattcctcgaacacatcaaacccagtcgcagggcttttgtacctgctattgtagtcacctggagggttcttcccccagttttccaaatggcttaccccatctcttcattcgggagaggtttttcctgaccagtaaccccatacaaaaagctttagttttctttaaagaacttattatctgatacactacatatttattttctgggcccctcaccagaatgtaaatttaatcaaggtacagattatactttattgactgatatatctgatatatcactagaggccatcacagtgcctagctcagatccagatgtgttctcaacaaatatttgttgaatgaatgaaggaagctattgccatagcccaaaaaagctcagaataaagcagtggtgaggaagagagagaatctaggagatatgaagggatcacaccctgctgcctgcttttctctgactgcctctttccaaggaaactaagctgggggagggaggcaatggcaggcaagagacatttttaagcctcttggttgtagaggagactgcaagagataaattgttctttcagccttgctccagtgaggtctccctgcctccgtctgctcactggtttctgtgcctttttcatctcccctttggctgagtgctggcagcattggtttgctacttgcagtgttaggtgcctgcttagaaagtctgtttagttcaaagagttattaagcatgtgccatgtgctaagcattatgataggtacagaggagacagggaaagagagacctcagccaaggagctgaaatctagggtgggaaggcagacaaattggaccattttcctgcaatgtagtaagtgctacacagaggaaagcccaaaagaagggcccttaatccagatgggaggcagttagggaaatagtcttaggagaggtgacactagagggtaaggattagtaatgggaagaggggaacaacatgcacaaaggcagaggcatgtgacagcatacaacaagagtcacagacaatcactcttataaaagcaggaagtgcacattagagtctttgacaaggttcattctagaagtattgggaacataaattgagggcttcacccagaaaacattcacctgtgccccacccactctcacttccctccagtgtcctgaacacacacgtacttctaccagtgggatttggctggtgccaaagtgccaagtacataaggggaaggcaaggagggtttgtcctagcccaggaagaatgagcggacttctttgctctgaggagagctgaagtattgaccctcccttccccattaacccatatccagctgccacccaaggggaagcttcggagcctgtgtagccagcatgtggaaaggctgcagatcttccagcacctccaccccatcgtggtccaagccgctttccctccactctacaaggagctcttcagcactgaaaccgagtcacctgtggggctgtccaagtgacctggaagagggactccttgcctctccctatggcctgctggcccacctccctggaccccgttccaccctcacccttttcctttcccatgaaccctggagggtggtccccaccagctctttggaagtgagcagatgctgcggctggctttctgtcagcaggccggcctggcagtgggacaatcgccagagggtggggctggcagaacaccatctccagcctcagctttgacctgtctcatttcccatattccttcacacccagcttctggaaggcatggggtggctgggatttaaggacttctgggggaccaagacatcctcaagaaaacaggggcatccagggctccctggatgaatagaatgcaattcattcagaagctcagaagctaagaataagcctttgaaatacctcattgcatttccctttgggcttcggcttggggagatggatcaagctcagagactggcagtgagagcccagaaggacctgtataaaatgaatctggagctttacattttctgcctctgccttcctcccagctcagcaaggaagtatttgggcaccctaccctttacctggggtctaaccaaaaatggatgggatgaggatgagaggctggagataattgttttatgggatttgggtgtgggactagggtacaatgaaggccaagagcatctcagacatagagttaaaactcaaacctcttatgtgcactttaaagatagactttaggggctggcacaaatctgatcagagacacatatccatacacaggtgaaacacatacagactcaacagcaatcatgcagttccagagacacatgaacctgacacaatctctcttatccttgaggccacagcttggaggagcctagaggcctcaggggaaagtcccaatcctgagggaccctcccaaacatttccatggtgctccagtccactgatcttgggtctggggtgatccaaataccaccccagctccagctgtcttctaccactagaagacccaagagaagcagaagtcgctcgcactggtcagtcggaaggcaagatcagatcctggaggactttcctggcctgcccgccagccctgctcttgttgtggagaaggaagcagatgtgatcacatcaccccgtcattgggcaccgctgactccagcatggaggacaccagggagcagggcctgggcctgtttccccagctgtgatcttgcccagaacctctcttggcttcataaacagctgtgaaccctcccctgagggattaacagcaatgatgggcagtcgtggagttgggggggttgggggtgggattgtgtcctctaaggggacgggttcatctgagtaaacataaaccccaacttgtgccattctttataaaatgattttaaaggcaa

SEQ ID NO: 2 - DNA, 25483 bp, Mus musculus
aggtgctccctccctcttccctcctccctcccttgggccctgctccctgccctcctgggcagccagggcagcaaggacggcaccaagggagctaccccatggacagggccccacagagacaccaccggacatctcggggtaagagaccctaaagccctgcaggcaggtggaagggactgtcagggggctcagaggaggggagggaggcgaagagactgggaaagaaagaactggggagaagagaggtgagcagaggggagatggactggcagacagagcaaagcggtgaggtaggaccgagtctttacataactgtaggggggggacaggaagagggcctagggtaacagcaggagacctgggaagacggggagggcaagaaggaagagacaggttggagtgggggcaggagggaggagctgtgttagggaggcttgatcgagaggatgggaatggggctggctcccaggtgtgagcaggcccctccctgcctgccacagaaccctgggcagcagcggctggaagggtgactctccgccttcctattcattcacaagtggctgccgttctggcgcaggggctgggggtgggggacctgggagagaagatgcagttgcaccatgccagctgctctagcccagcagtcccacgctttccttcaagctggtccgagcacggagttttatctttgctgtgtgaggcacctgtggagcacagaaaggaactggggaacagtcccccgatggagtgaggagggagcccttcagaacaggacatcccctccctccctcccatgcttgtcagctgggaacctagagagagtgaacgacagaagtgccagcttctagggccactagagaaaggctccggggtgggagtgggagtgggggccaacaaggggagtgtccccatgcaagactgctctgaattgcaaagttggaggctggacaagggtgccacgtcagggaggaaactgagtagggccagacaggattagcagggaggtgggcatggcatgaagccacaccctctctgggcagaccttcccctcccccacccggggaacaggctaccaggccccatttactatcacggcaatgaaatgcaggaagcctggctgcagagtgcatctcctggcagagggacagtgaaggagggacaggacatgtgtgccaggcttggacagcagaaggcaaaaagtaacagaaaggaatcaaaggttagggacattacagacagggctaatgggctttctggaacagaagactggccctaggcaccctggatataggaaatgggttgcggcctcttttgccaagggctccctctctaggtgtttcccaaatactgactgcatgctgatttcatcccagatatgtaaacagccctgtaactatgcagtaaccatgactctcccctcagctgctgctcccctggacagcagagcatctctgtaaacctccacgaaccatggggtgcctcctcctgtctgatctccacccagacccatccacgagcaaagcagcaaggcaaagggatcttccctctgcaggcttgtgggcaggtgaagcacagtggcggccagagagggtctatctgcagctcggccctccttgtcttcctcttcgcccaccctccccatgcactcccagccccacacctctgcagctccctcttgctttcaggcacagataagcaaccaaaagactgcattccctctgggtgcagaatatgtgtgtacgtcaaatgcaccagatactagagggttcttgctgttccccagagcaacaagctgaacaagacagacagaggctctgtctccagacgggcttacaatctagaagggatgatggcatacctagggcagttgtctgttatgtcaagtgccaggaaacaatgcagagtgctggctgagtaaaccccagggcaggggacagggcatgggaggctgccccagaggaaaagagagacatctgagatctagctaaatgggggagggagggtagagtgtgacatgaggaagtcctggaggcagagaggagctgggcactttcaggacctggaagagggccagtgtggccaaagggcaaagtgatgggctctgccaaggggcccagcttctcagaggccaggtagtgctggggtaaaaatggggcagggcaggagccaggaactggggaagtctttggcttttcccctaacatcttcaactattcactgatcccttccttctctttacagagctgctggctgcaaagaagacccacacctgtgagtaggggtttgggccaagaaggtggcacggggtatggcaaaagcattcagttcaggaggcatgagtgaaagaacacccgggactggacagaattggaagaatcaggctaagactgcaaagcccaagagataagggccaaagggaaagacttataggcttataggccaggaccaaaaaaaaaaaaaaaaaaaaaaaagaagcccaaggggtgccaagttacaagcatagaaagaaaaggggaactgggaaagaggagggcagggtgctggacagaggctcagctgctgtgtctgaccagggaggaggtgaaggccaccccagcctcagaactcagcagccacaataggaggcctgggagcgtgcccagggctttgtggtggcagagccaggtttggtgttcatctctgtggttaacacattctgaggtgtgagcaagcctggagagaggctctgcagagctagagagtaggaaagccttgtctctgtaagaatgagtggacaggaacccgaaatcctcagactgcagtgtacgaggaagagaccagagttccagaagggcttcccaatggacacttgcaagtaaacatctgtctcaggccagtgcagcacccccaatccagccacatagagagaagctattcccctacaaaatgtgcccgctccaccaaagtcctccccaggggttcgtgcataccctcagcaccttgggggcactctggaaaagccacaagcatggtcattaagttaatagtgacaatctcatcagaggaggtcacctctactcttccatcacatactcattggttgcccaccaatctgtccccactacaaaagccatctgtggccttcctgtcccagcatccctcctccctgagcttggggctccatcctcctggggggggtcggagctgcttggctcagcataatcctgatcagcctcctgtgcactagccacagggccccacggaaacgctgagcagggccctgggaggaaagcgagtcagaatgacgcaggcaagctgggggaggggaccagggaccacacttgggggtgtagagggggacttttggagagtggaaactgggagagaccaagccaagcttttagacctgcctcccatcctttaacccttaccatgtgtcctcctgaggatccaggctagttaccctcatccatccaatgtccaattcccaagctcgcagagagagctttttactaaccagaaagattgaagacctctcaaggaggttgagctccttgagtttttattgtcttggccccaaccccaggccaagacaataaaaactgcctcccaagtgaaataacctcaagaaaggggtccaagctgagaaacccgggggcacacccagaccaagaggggaccgaatgactaaggggccagaagaggaacctccaaggctgaggtaccccacagagcagatggaaaacaaatgaatccatcaataagaaatctcacaccaacaaaacctgaagagaaactcaagtgccaggagacgggccagtctgagacacactcgaatgcaaacctgaaccagagatacccttctatccctccagtggatctgaggtcactctacctggccataagtccttactcaaccattcactactgtgtgatcttgagcaggttacttaatctctctgtgtctcaccttccttgtctttggaatggtagttatcacataaagtattttatggggattatgaagtccacacagagctgaatcattcccaacactgaattaagcactgctgctaagaggatgaagatggtagtgtcactatctgtgtcccagactagcagtcttgtttccaaaggcctttctgaaggaccaacccatcctacagatcctacagagggtatttgcctgatgatactgccgctatcgtttcctcagcccaggatagcatcatgtgtaggaggaatttgggtgtggtgagggcagcctcccggttgtaccacactggttatggctgttgacagtccacagggtctcagtgccacaagacaccacccaagacagattcctgttacttacctttggaacatccctacccctgatgtcacttggtgaagagggcctggggtactcaggagaggggatttcgagcctggcctctgcccatgagctccacgaagctccccagctagaactcccctggcgagtggaaacagcttttaccgcggctgtagctgtggttttggaattttccaacgccccctgtgattggctgccccgcccctcacaccctgccccagacccagattggccacgtggggtgcctgtcatcatacccaatgcacctctgggggttggggggctgtcacttggccacctgtgtggagcagagcttaaacccccctgcccagaaacactgggggagagctttgtgcagatctaagggctgaggcacccgctgagagggcttcaccccacctccactgccagctgtgtgctgtcctgggctaccctactgaggaggacagggagccaagttctcagtcatgagaagtaagtgaatgggggcatccggtcatgggggagcctgggtcctgtcaccattcctaggcccgctgaataggagtgtatcttggaaaccgtgcctctttggcagggtgtgtcccagtcaaggtcaagatctgctgggagatgggtggagtcccaagagagttactcttccctggcagcttccttggcagcaatggtaatcaaattattgaggagttcctgacataagttctgaagttctgggaagactgagcatgcccaagggtccaaccctttgatttacaaagagaccaagacccaagaggggagtgcatcactgaagagctcaccattagggcctgggagctggtggagtctggtagacattaggacccacagcttatattccttgttcctagtgaagagtttatctttgtgcctccaactgcaggcactgctgtaccctgaggcaggagtcacagtaaactgaggtcagcaggcagtggggatcagaactcatcatctccctgattccctaaccttaaacacacacacgcacacactcataccagggcctgatggctcagtacaatccagctagggactgctctgtgtgtgctatgtgtatatttgtgtgtgtgtttgcatatgcttcaggtgcagttgatcatctatagcaagaagagatgggagcagaaaaccttggtctcactcctttccctgcttgaaaccatgggcccacagctgctgggcagatgtcaggggccctttaggcttccagctgagcaatgtgggggatccgatcctccctgctcatgtaagggaagccagaggacctctcaaagtctacagtgagtgaggaaaagggaagcctgttaccctgaggcctgaggaagccccagctttaacctggggtctttccacaagccacaaaaggggaggccatactgagtcctggaaaggcccatggactgaaaggctagtgagcaggttctaacacagggtcacctgaggcaagccgctgatctctggtctccagccacaaaataaatgccaagcatgggagtctctgagttctaagagcccaagaccaaagagaccccctcgtcccctaatgggtgaaagagaatagacccctatagtatacaaggtcaagttgggattccacttgcatgcatgggacaggactatagtccttggtgagacaagaggaccaggagaagaaccaaaagtcctaaaatggagtaggagccgtggttcttttctggcttcttcccctccgcagcaaaagctggcagatcgatttcacagaaacagccccaggtcggccgaagcagagggcaacagccccaatagtatctgagggatacacttgggtagctctgcgttttatgcacacatgcacgcgcgcgcgcgcaaacacacacacacacaacacatgcatacacataaatatatccaagttttctgacccctttgaattccagttaccacctacttgggagaggtcagagcagagagggtttaggaccatgacacaccaaagagtgaggccagagaaacaaggaatagatggaatgtaggaaataagcgatgggtttgagggtcaagggggaaggggtccagatggagcactaccaggagagccatagagtaagaagtccagagacgaagggcacaggtcataaagtacagacacgggaggtgggaagggaacatggcagactggagggtgtctcaggaagaaacaaagccccttcgacccctacctcggccagtcaatggtgtatgacatagccatctcactgttaggagctagtcagtgtggaatcagtagacaggaagtctaggaatgggaggtcacatgccagtcctcttccttgaatacagccatgattatgttgagcaacgggccacaaagagctccgagtccccagggtgtgtgtgtgtgtgtgtgtgtgtgtgtgtgtgtgtgtgtatgtacattcggtagctgattccttccttagcaatgctggaaattgaactcatgccacaggcctttgtggctagcactctcacccaccgagccttctcatgggccttttatttggttttgtttgtgacaaaatgtcatagactggctttgaactccatatacagctgagagtgaccgtgaattcctgatctgcctgcctctgcctcccacgtgctaggattgtaatatagagcatcaggccctgctccatcagccttgttccttccttgtatcaatcactcctgcatctttctcttttcctttcttcccattcctacccagaatcctgactgtcccaggctcaagattctaggatgtgaagatcttcaatctgttccatcgcaatgaatatgtgtcttgataactgctgtccctaccaggggctcacccacccctccctcccctgcctctgttgctgactcaaaccaacagggacagggactttccccatgctgagtgctctctaaggaagacagcctggggtctcactcctgccccgtgattatttcctggggtctaatctccactcctgctgcaatgatgacacggcctcttccctgagactccaaggctcaaagagtggagttctgtttgggagcagaacagaaacaggcagaatttcagtaccacagccaggtcttcctgagtctgcgtccctcccagaggcagagccagagctctggaggcaggcaggcaggcgaggctcccactcctcagagcttcttcctcctggtgattcatccccttcccccatccccggcttgttttctttgcgttcttttatttcctctcctttctccagtcccagactgtgggggtggtgggggcagcaagagggggtttcgagtggctggctggctggcttgctttcttggctttgcaaaacctgtctctccctcgcccacctgagttttagagtcaccagtttttcagttctgatatcaggtatgtcagtagaaaattccatgagggcttgcctggttggggacatgcccagcaggtaaatcagtggttcctgtccctgtggtggcacccaccacctgggtttccagcagaaactggaggaactgagaactaaggaatatgggaggctgatgacaggttgtggcacataggggaccactggctggagctgtggtctcagtgaatagagaaggggcctaagctgagagatgcattttctttctcatccagccattcactcactgatgcaaagaaaggcccaacaaggggcaacctagcccataccctcaaggagctgtggacttccagaggagccctgggtcaggagctctgctggggtgcatgggtcatgtgatcttggctctagagaagtagataaagggtgcatgggccagccaggaccactgagggaagccaggcccaaggaatggtatctgtctgtcggtttatctatctctctacctatctacctatctatgtatcatctatgtctcatctgtctgtctgtctgtctatatctttgtacgaggcatgagtcctggtttattcctcacctagcctatcattacccttgtttcacacttgatcattttgcagccaatgaccttgctctatccgctctcttttagtatacttaggtatctcatcctccaaggggatacagcttaatgattgaggactctgactccagttaccaaaacctgaatgtaaactccttgcttgccttttcctggctgtatagactcggtctaatcactctctaggcctcagtttttgtttttttttaatctgtaaaatggggacaatactaacagaccctactttacagaattgttctgatgattaaaagtatatgtaaagagtcctcaggacaatggaatggtactgcaggaccttgccttgcaatcttggcgacttgaattcaatctccagaacccatgagaaggtaaaaggaaaaaacagatttcacagagttgtcccctgacttccacatgtaagctgtggcatttgtgcccacatgtatatatagcatgcacacatgtagtataataattcataaattatttttttaaaggaagctgagtgtggtggttccataatcccagcacatgggaggctgaagcaggaagatcttgcatttcaggccagcctgagtacgcagtgagaccctgtttaaaagaagggctgggaggcagtggggcagctcagtggggaaaggcattgctgtcaagtttgataacctgagtgcaatgcccaggcctcacatggaagaaggagagcaccaatcctagaagctgtcctctgacctccacacattcaccgtggtgtgtggctcatgtgcaggcataattaataagtgaattaatttagccaggcggtggtggcgcacacctttagtcccagcactcgggaggcagaggcaggcggatttctaagttcgaggccagcctggtctacaaagtgagtgccaggacagccagggctacacagagaaaccctgtctcaaaaaaaaaaaaaaaaatttagttgaggctgggggaatagctgtcctttcactctgctccctttgtgcccatgggctggtgggcagtgacccctgaggaaaggggagacccacacatgagaccttggattgtgtcccacagcacagcacaaaacacacacacacacactgtaaagcctggcatacactaaaaattcaggcagtgtctacatcttttgttattcttccttcttactcagtatcagctggaaagcaggaaaagaggaacagaagagagccctagcatgcctctgcctaaaccattccttccctgaaactggggcttctggagtgagaccctcctgggctgtagcccctctccgttccaaccacttcctctctgtggctaggcacctggtcaggacccagggcccagctctggatatagttaaaatgcactatcaatgaatcttgcagctgtgagcagcgtgagattagaggaggttgggggcagaagtggcttgcttctaccgtatttctcctccctggaggctctaaggtgctccttgaagagcgtttcagggcagaagcaatccaaaggagagtcacttttgctttccagggctgcaacataattatagtttttacatcacatccgtagggaagatgcagagataaactcagtgagctgacctgtataaggaatgggtttgggaagtgattatcaaacctaccttgacatcttgggaggagcagcctggcacaaaagcagccagagactaaaatgtttttatgccaagcatagtctgaaggcaaagaatcactgtcctggagtgcattataagtgtggactttccgagccctgccttgggctgcttgaacaaagatcttcatggtggtggtggtgttgttgttgttgttgttgttgttgttgttgttgttgttttgtggtactgggccatggaactcagaacatgtgtatactaggcaagccctccactactgagctactgctgtagctatatttttaacaagaccaggtcctatattttaacaagacctccaggttctctttttttgaaagacaaaagactagagttgctagctgggtgcctcctgcaccaggcatttctgcttttgtaagaataaagatagaggggtttttttttttttttttccttctttcagtttttagagacagagtttctctgtatagccctggctgtcctggaactcactttgtagaccaggctggcctcgaactcagaaatcctcctgcctctgcctcccgagtgctgggattaaaggtgtatgccaccactgcccggctggttgtcatttttaaaacagggtctcaaactatacgccaggctggcctgaaactcatggcaacccacctgccccagctttctgaatgttgagatttcccagcttgagggttttctttgtgatacccttcaggagaaaggcacaatgagggaacagtaagacacaaaaatcctaagaaagaagcagtttggctgctgtgggagccatggggcttgggctgacctgaaggctcctgacctttgattggctccagttcctggcaccgttgggccctgagatggtaagttcctggcagactaggctcccaggcaacagtttgagtaatcctgtgattactcagcaccccctccccaagcggggttcccatcacctgctgttcagggtctgagtcttgaagctttgctgtggaagatgtttctccgctcctctcatgctgacttccctaccagcccttcccctccttccttccccaagtgtctgtctctctctgactttgtttgtctgtctctgtttgtctctatcttcccaccacacacacacacacacacacacacacacacacacacacacacaccccactggtactttctttgatatttaagtgtttagggtggatggtactgaacagggtgaaggtgtaggggacggagaactagagaaagtcaagaagtttggtcatgtggaggattgggcacaggaccagaacaagcaggggtttcccacgatttcagttgtctctcctttgctataactattttcccccagtcctgaatctctcagtctccccgtttcttgtgcttgtctcattgtagaccactgctttggattggcaatgggaagatagaagaggggctacgctggtagctagggtccagggctcccatagcccccaaactcccagttcttgactggtcatatctcctatgagatggcagggtcttacttacactgtggtaaggttcctgggttaggaccagcaatgggtcaggtatggggcaggaggtatgactggggtcatccatgcggtcagtgtacacacgcacacggatgtggctcttggagaagggaagaggtagggaggcctgtggttgcctgctaggccagggcctgagttcccaccgtggcttggcctaatctccctaccacttgcttttctgggtgacctatgttggtttccccctctctggtcttagggccactgaagagtgatataccacagagtacagaggagaaggtgttgggtaggagcaaaggctgtggacccaagtgttactgccaggctgccattcccatggatttgctttatctcagacagtaataccctgccctgtagtgctctgcctctccacggtgctccctgtactctcttgaatcatgccatgtgacctacaccacaggcaatgttgctttcaccgtcatttgctgccaagggaactgaggttgagagtgactggaagtgtgtgtgcccccacattttccacctctcttccaggcactcaggtcccctcctgttctctcttccccaccaagcatttaacccagcttgtaacttacaggaagccattgaacagagcatttgatacctggtggctggagcttactgtgcagttggcaggtagaaagtatgtctggaggtaggacaaagaactgagttttaatggaaggatttcaggcactcatatggccaatcccttaaagagacagctacttaatctgacccagctctgggctggcttgagaaggtcatagtttaaggatgatggaatactttgggaagtgatgggcaaatcatggtctaaccattccatatcagcagacctatgtgtggttatagattttggacatctcacatagccctggttagccttgaactcatgatgtagccaaggacaatatagaactcttgattgtcttgcttctacctcttaaatgctggaattacagagacgtagcagctctcatatgacagatgctaggcacaggctggacatgagatcctatgtgagtttgctctccatgaggcacttcctctgtccctagggtgggagacaggtcacagatgagatgggactgttactctagatctcttttctagcctgcttcaactctcgactatccactcaggaaaatccagaagtcagtcagtgattgggagaagagccagctcccccactcccaccctaccccttcgccccctagtctttggacttgttgatgaaaagatctggggtggctggaaccccaagctttacctagctgctgtcccttctccctcccaggtccccaaagaactgcagattgaacctggggcttcatgcatgctgctttaccacagagctaagtcctagctctttttcagttttttgtttgtttgtttgtttgtttgtttttcaagacaggctttctctgtgtagccctggctatcctggaactcaatttgcagaccaggctggccacaaactcactgagatccatctacctctgcctcctgactggtgagataaaaggtatgtgccaccactgttgccttggactttagtgtccaggaatcaagctctaaccaacaaatgtgtgtatgtgcactggtatagacaatataccgccaatccacaggccacagagaccaacctaccttcttttctccttccttccttccttccttccttccttccttccttccttccttccttcttcttgagcagtcctggctagcctggatcttgatatgtagatcaggcaagtcttgaactcaaagtaatctacctacctctgcctggctagtcctaggattaaaggctggcctcaaactgacatcatttcaacaagccacatatacttttcttctgtgcacacacacacacacacactcaagtatgcctccaaacatgtcaagaagataacagataatgaactgttcaagagagtggggttgtagacctggcactcaaagaaactagctgtgtgagcctgtgctaggtagttaggtcttcatctgtgagaagaacaggtggatggagtgtgctttaatctcagccagttttaacagtcgtgtcctgtgctcatacacatagacccagatgcctttgtacatcctcttacacacttacacagagcattgcctcgtcttggttctggggtcatcagtctagaaatcttatttgggctttaagacaatcagcaaagttgggttgagcccttctctagatttcatctgtttctttctagtctctctgtacctgctgtgttggttcccctcagttcctgtccctgtgtagccttcactttcctccaagagtgactaacatctctgtctagtgctcagtggctgtgccccatactctgttctgggagccaaacttcaatggggggaaggagacaaaatagaagccccctgggcgggaagcaggtgttacgaagcagtaaggcctcctctggccctatacaggatgagaggagggcactgaagatgttcaacttgaaggactgagcaggtggcctctttgcagctgctctctgtctccataaaagctgatacaactcccagctgctttgtgaacaaaacacagcctcctcagaccctatgctgagaatcatttacactttacttccccttccataatgcaagagggcgtgttggagctcactgaagaagtggggggagcaccatacacctgcgtctgcagcccaggctcatggtagtgaaatccagaaaaaaacattatgggctagcttctctttctctcttccagcacaaattgaagtgatcccttgcaagatctgtggggacaagtcatctgggatccactacggggttatcacctgtgaggggtgcaaggtgagttgtacatatttgtctgcatacatgcacttggctgtttcagcggtctccccagggtcaggaacaggagggaggaggaggacctaatctcgatgtaggaatgtgatcacagggtccatcacaattatacagtggaggttcggggactttggtggatgtagaaattcttgagaccagtgcacatgaattggaggtccctgggaccacctcaaactccgagagggtgggataagcagtttctgtttcccagggcttcttccgccgcagccagcagtgtaatgtggcctactcctgcacgcgtcagcagaactgccccattgaccgaaccagccgcaaccgatgccagcattgccgcctgcagaagtgcctggctctgggcatgtcccgagatggtgagaatgtgggggcagcccccaagagtccctgtactctccagagacatcctggctcttgccagagttggcttgcaaaaacagcctgtcaggggcctctttctgttcttctacccacagccctttgtcctgtctttttgagggtcctcaaggctcttcagcctctactccaggctctgctccagaaaacctttaccagcatcatcttagtactcttgtcccttcttcctctaatgagttctcttcattcttctttctcctggcctagttcctatccagttcccacactgttacctcctgccttgtttagctccatctccctcctgagtaactatccttaggcataggattgtggcaaggaacaccgtctgggttggcttgagaatgacccagaaggtgggggatcgagtgtggtgttcctcgagccgtatccacctcctcacccacctcctcacccaccgtcttcaccacaggaggagccctgggtggagtggggggcatgaggtgaggaagacccagaaggagcctgtcagcacttttcagtgctcaaaataacaaagccaaagcgaaaggaaacatgcaggggtgcaaaggggcaggcggggcgaagggctgtgcccccacacctgggaggggttgggggagtgaaaaggcaggaaagagagagcagaagaggatgttcagaagcaagccaccagagcctgggttgggctgtggtgagtatctaggtcaccagggagcctgcaggcctgaccacagggaaacctgtgttcgcagcccttctcttcctccagccctcccagacaggcaagctgaccccaatacagcctgaggccccttactcaacccccacctcagccctagtctcaggagactcgactccccggcccaagcccattgcttgagttctgcactattagcatctagtctagagctgaaagcattttgctggggagatggaaatgctggtggaaccgatcctaaagagagcagagccaggcatgaaaggagcctggagcctaagctccccaaaagaaagctcatagacagagctggggaaatggagcatggagtcagattcatgtgcctgttgccctgtcctgtcttgtcttctcttacctcctgtactgattcctgaaccttcttcagctgtcaagtttggccgaatgtccaagaagcagagggacagtctacatgcagaagtgcagaaacaactgcaacagcagcagcaacaggaacaagtggccaagactcctccagctgggagccgcggagcagacacacttacatacactttagggctctcagatgggcagctaccactgggcgcctcacctgacctacccgaggcctctgcttgtccccctggcctcctgagagcctcaggctctggcccaccatattccaataccttggccaaaacagaggtccagggggcctcctgccaccttgagtatagtccagaacgaggcaaagctgaaggcagagacagcatctatagcactgacggccaacttactcttggaagatgtggacttcgttttgaggaaaccaggcatcctgaacttggggaaccagaacagggtccagacagccactgcattcccagtttctgcagtgccccagaggtaccatatgcctctctgacagacataggtgagcatctgggaagggtgggggcagtgaaaatgagacaagaacttcctccagcacggtgcccatgtaatcaagcattagtcctaaggaattagggatcctggacaaaaagccaagggaggaggcagagcaagggaggccaggcagagggcctctttatgaactttggggtgggaactggctgatatctagctgtgacttcatcttctggccccagagtacctggtacagaatgtctgcaagtccttccgagagacatgccagctgcgactggaggaccttctacggcagcgcaccaacctcttttcacgggaggaggtgaccagctaccagaggaaggtaagggcaagagacatgagggaagggagggcaccaccacacgcgggtgcggtgcgggcgcgcgcgcgcgcacacacacacacacactggtagagcccagatatggcgtctttcacaggaatgggggtagcaatagggtatcacaggctggctaacaggtgtgactgtctgtatccaggcagcaagatgactatttctgtagctcctgcttattgagatttcacctagttagcaacctacatcctcttccacccagaccttgccacactgcctttcatcctccatcagtaactgatgctaatcagtatctgagggtcatttactggacaccctttcctgtcaggcattgtaatagaagctttgaattgtgttcaacctgctgtttgtgaactacaagtgtctaaagatagtgataaatgtggcccaatgcaaaatcatgagaatgtttttggttggttgattggttggttggttggttggttggttggttgttggttggatgttgttggttatttggttgtggttggttgttggttgttggttggttggttggttggttggttggttgattggttgttggttagtttggctggttccaagacaaggttttgctgtgtagccctggctgtcctggaacttacttggtagaccaggctggcctcgaactcagagattcacctgcctctgcctcctgagtgccggaactaaatgtgtgcactaccaccacccagctctaaaatgtgagatttttagaaacttgattctcaggtataaactttgtagataactatgtcaaattacagtgtcagaggctagacacacctgtgagatcatcctcagcccgtccaacaactggcctctgagaacagaatttacactgagggagaagtacagaagatcatacagagatggctccacagtgtctgccaccccttctgtcacactctgacagtaccagaggctctgaagtcagctggcacttcacatttgcacctctcagttgctgagaccttcttcaggaggagcagtaattaacaatgtgtacactgtttgcaggtgaaactgtatcatgtatggtttccctttctccacaacagctatcacagtgttgcaggaaagccatcgcctcctatctggagccactccctgggaatccgggaagctctctggcaaccttttctctcccgtagcagaatcctaatacctagtattgaatggacttcacaagagaccaggttatcagggagaaaggagtttgaagttaagaaattagaagttttcaacccttatataagtctctgggattccttgtactgagctggggatagcagtaactgtaactcactgacaggcactgaccctggctacatttgtgctaataggctctatggttgacaacaatatacaactcataccctaaagtttatggggtgcaggggcttggggggatcacaggtctcctcctctatccccgcagtcaatgtgggagatgtgggagcgctgtgcccaccacctcactgaggccattcagtatgtggtggagtttgccaagcggctttcaggcttcatggagctctgccagaatgaccagatcatactactgaaagcaggtgcacagggattggcaggccctgggggtgggggtggagcatgggctggggatggaaggacagacccagggccaagtggagggaggtgacttaaggaaatcaagacaccgagggcttaacaagacactggctctgcttaacatggcctacccatctttctcccctttatccaggagcaatggaagtcgtcctagtcagaatgtgcagggcctacaatgccaacaaccacacagtcttttttgaaggcaaatacggtggtgtggagctgtttcgagccttgggtgagggcagtgggaattgagaaagtcctgatgccaatcctatcacaagcctctctacatggttgtttgccccctgctctaaacacccaagagtggcatccttgggggagaggggaggcagctaccatgcttactctcttcatctccactccggcaggctgcagcgagctcatcagctccatatttgacttttcccacttcctcagcgccctgtgtttttctgaggatgagattgccctctacacggccctggttctcatcaatgccagtgagtgtggctgggcatgggagcgggcactcgtggctgagacacagcagctaatggcgaacctaggcctttggatgtgactaatgggagactgcttgaaataaggaaatgagctctatcccgtgcttctgtaaaatataacagactaaagtatgcagaggaaccttaagacagggcgaggatagcatacagtggggcagtgggaacatggagaagggaggttggaaggaaatgagccacttccccaatagatgttaacctactagccagtgtagggcagtgactcctttacagtacacatgggaatcacctagggagctttaaggactaattgagtccctgggtcccacgtccagattttgacataactcatctaggctgcacccaaaattttaagtcacctccagattgagccactaagactgagaatggccacttgatgtgagctcattttgggacagaatgcctatactggcagtagagctctgggtccaagcagctgaacgataaatattcagaggacctaggggagtgggcctgctgctctgggttggttaatgaccatgcaagccttccagctctactaacatgacttcaagctagaagcaagacttctagcaaagggaaaggtagcttaggggctgaaagagagccactgagtacgttagagtccttggtaagaaggtcacctctctgagtcactcctgtaggaatgaggaagctctcttctaacattttacttccatgacagaaatctagtgcctgacattgaataagctacatgaaaggcaggttaccagggacaaggtagctaaaagttagttaggagattaaaagttagttaaggcttgtatggtcattaaccatcccagagcagcaggcccactcccctaggccttctgaatatttatcgttcagctgcttggacccagagctctagtgccagtataggcattctgtcccaaaatgagctcacatcaagtggccattctcagtcttagaatgtctccccacccctttcatctctgcccagtttccctagtagttagctcgacaggcctagagtcatacagtttgctgtagtcaaaccagtacacacatgtgcgcacacatgcatgggggtggggtggggagggacagagacacagagagacagaggcagaaagagacggagacagagattctcttcaaaaagatacatgacaccattttgttggtcacgactgtctttgttgtttccgtttcactctggtcccatcccatcccttccttcagaccgtcctgggctccaagagaagaggagagtggaacatctgcaatacaatttggaactggctttccatcatcatctctgcaagactcatcgacaaggcctcctagccaaggtaggagcagtccacagggtagaagaaactaggcccactgccagttgtgtgacatcagggccagggtcttcgggtgcagaggaaggagtgctgcagtgctgggctatgtcagcgtttgcagcagctgtgggccctgctggagcatctgtttccatgtacgaagggatggaaagttagtgtggagttagaagagacctccagggaacaattcagtttaatatagctgacacttacccagcacctgcttatacaaggaactgtggaaagctacagagatgcagttcttgtccccactaagatattctaacctcttaaaaagagacttgtgtaccttctaatataatgctaatatggggtaaaatatgtgatattttaacagtgaggttaacaaagtgctttcaatgatatctcttatcctaatggcaaaccagttaaaatagggcaggtgttagaatcttcctgtagcaataaagtgactccagtgacacatattaattgataacacaaatcttaatcccagtgctctctcaacaacatccccagggcccctaatttgctatttaaaaagctcttagaagcacgcctcggttgtgcgtgcccgtaataccagcattcaagaggcagccgggagcaagagaaacaagaatccaaggtcatcctcagctccataatgagtttcaggcctgcctgggctacatgagatccccccttaaaaagtgggggctgcttttgagaaaatgacagggtttcaaggcaacttaaggggctggtgagatggctgaatgggtagatgcttgccacaaagcctagcatgatgagctgagtttaataactgggactcagatgatgaaagcacaaatctaactccagcaagttgacctctgaccttcatacacatgtctgctcacaagcacacacaaatataaaaatgtaaaaattcctcacaacttgaaggtaaagccagtaaaacataaatccttcctttggggtgagagaatgagaccatgaaatataccggttttaataaacattcctgaagtggagcagggatccaggcttagggaatgggatgaatggagctctgaggagaccagatagtacatgaggaatggctcatagctcatgtttccgtgtgtgtatgtgtgtgtgtgtgtgtgtgtgcactcgtgtgtgtgtgggtgtgtgtgtgatcggttatgtgcatatagatgcttctgcatacctgtagaggccagataatctcaggtaccattcctttggtgctgcatttttatatttttcatttgttcattcattctggacagggtctctcatagtctagcccggcctatgagtgacctaggtctgctgagtcccaagagatgatttgcctatctccacatctcaaatgttgagattataaacatgtactaccttgtctggcctctctctccctctctctctctctctctctctctctctctctctctctctctctccttccctccctccctccttccttttccttttccttttccttttccttcttcttctttcttgtttttttttttcttttggttttttgagacagggtttctctgtgtatccctggctgtcctgaaacttactctgtagaccaagctggccttaaacttagagatctgcttgtctctgcctcccaaatactgagatcaaagtcttgtgccaccacatccagttttcacctggttttctttccgtgggttctgggatctgcattcaggccttcatgcctgaaggccagcacgttgttgaccttcatggtacttttggtaaatgtgaggtcagaagctggggtagactgataaagcagaagagtagcagaaggcagcctggaaaccgctggaggaagagcagttaggaaggctttcagtgccgtatgaagagtgaaagcctcacttctaggcaatgctgtactcagagctgcttagggaatttccttctgacctgtgtgaaggatccatctatgtaaccgttcgctcaggcccttgttattcacagtcatcacaggagtcctgagatacagaaatcacttcaaacagtctctccctgaggaatgtaaactttaatctacaacaaaatggatttaaagaaggtctgggaaagcagttggaatacaaatgtggttggatccactttggtgccttttgttctgggtttttgaggcagtttcatgaagccaaaggtagccttaaactcatgatcctcctgcctccagctcctaagtgctgagatcacagccatgtaccactttgcccggcagaatccactttcaaaatatatcacgtgtcccatgatgtgccccccccccatccagctatcagccacaattggactattatactcctaactcaatcccaccccatctttgtctgccacgtcagagccacacagcacttgctcagtaaccaccctggtcattttaaggagacaagacaaaacctgcctcttttgatctccagcctcctattttagccaaaatccaactccagagtccatgttacagtcaaatggaccaccctgccttcctcctcacctgacgttgcaccatcctttgactcccctactctgaccacagtattttttcactggtcccatctctctggggcctcttatacctgctattgtctcctgtcatattctcttccctgtttccaagtattttctccaggccttcattcaagagaggttttccttaaacagttaccggactggagaaggaccccatcccttatcctgctttagtatcagatacaatcatatgctgcttactaacaggaatatgttctaagaaatgcttacccatagcttcacatggtggggtacaactggatatacttaatacaaacaaacacagctgtactgtcgtccatactcccttagccttatgggaccactgaagtttgaggttcataattccccgaaaagttgttaggcggtacgtaactgtgtttatgactccctggctgctgtgcacatttaataaaagcacatctttttattcaccgatgttacaccagagctcatgacagtgcctcatctagatttatggagtttctcaacaaatatcttttgaatgaataaaagaaactattgtagtaacccaggcaaactcaaagtactaaaacacaaaataaattcaagaggcgtaagggactcactctgctacctacttttctgattgttactttttctaaggaactaagctaagaaggggagatgtcaagaaagagtggtttttaagtctcagttcattatgctgtaaattgcgtaggagagatggtgcctggggtctttctccctgcctctgtcccctgggcttctgcacctttcttagaggtttaccttcctttggctggaggcttactatactgacttactacctgctgagttaggcaccttcctagaaactgtttagttaaaacaagcaggtgatgaacatgaattcagcattcatgccagggacagaagatacatagtggcaaaaagacagatggactttatctaagtacatgtggggcaggaaggcagacagactggatccttttttctacagtgtggcaaatgctacacaaagggaagccaacaggacttttgcccagcaagggatggggatgatattctcagaggagataacacttgaattagcaaaataagagttagcagagcctcaccctccagatgaagaaacaacatgaaccaaggcaaagggccatgggagcaaacacaattcattctggggtaggcagagccattgatgccatcattcaagcatgtccttgctccaagcacagtcctgaaggtacagaaatgaccatcaaaattgaacctaggaaaagctcacctgtctcgtgtcagttctaacttagcctgaggtttccagatatgcatacatctaacaaatgggattggctgctcaagttgggtcaagggtcggggaggcatcaagaagggtcatcctagctcagtaacagtgagatgtgtttgctctgctaagcaccgaagtactcattccctcctaacctatcctcagctgccacccaaaggaaaactccggagcctgtgcagccaacatgtggaaaagctgcagatcttccagcacctccaccccatcgtggtccaagccgccttccctccactctataaggaactcttcagcactgatgttgaatcccctgaggggctgtcaaagtgatctggaggaaggacaactttctatttccttcagccctctgacccgtctccctggactcccttcacccagcctttccctttctgcactctatgaagggtggtatccctaggagtaagcaaatcctaagactgattttctgcccctaggcttgccttgtaggacaacagcagcaagtgatggagaaaaggcttgttatgtttgatttcccataagttccaccctggcttctggaagctgtggggtagatgggatagagataggatgaccaagtcaaataaaaaacagactgacaatcagcagggataaatccaggtacctgggataaggagaactcaaatctaggcttgaaagctaataacagtcctttcaatacctcattgtatttccccatgggtcctcctggggggacatggatctagctcagagactggtggcaagcccccagaaggacctgtatataataagaatatagattcctgagacttttctgcctttcttcttcctagttaagaaatgttgttgaccccctctgcctgttttctgggacctaaaatgcctggatgtgtaaagaatgagggtggggtggagataaggtcccaagataactgttttatggggtttgggtatgaagaaaaacatcactggaaaaattagaatggaaacctctttgcacactttaaaagtgtcagattcgttagcagtctaatcagagacacacatccacacaggtggagcacacagaggctctgcccccagtgacaccattctgtagactttccctctggcacacaatctcttccttgaggttgcagctctgagaagcctgaggttctaattcatacaggacaccagaattcatcccagctccagctgtcctctgtccctaagagaagcagaggaccggatactaaccagccggaaaa

SEQ ID NO: 3 - DNA, 1494 bp, Homo sapiens
atgagaacacaaattgaagtgatcccttgcaaaatctgtggggacaagtcgtctgggatccactacggggttatcacctgtgaggggtgcaagggcttcttccgccggagccagcgctgtaacgcggcctactcctgcacccgtcagcagaactgccccatcgaccgcaccagccgaaaccgatgccagcactgccgcctgcagaaatgcctggcgctgggcatgtcccgagatgctgtcaagttcggccgcatgtccaagaagcagagggacagcctgcatgcagaagtgcagaaacagctgcagcagcggcaacagcagcaacaggaaccagtggtcaagacccctccagcaggggcccaaggagcagataccctcacctacaccttggggctcccagacgggcagctgcccctgggctcctcgcctgacctgcctgaggcttctgcctgtccccctggcctcctgaaagcctcaggctctgggccctcatattccaacaacttggccaaggcagggctcaatggggcctcatgccaccttgaatacagccctgagcggggcaaggctgagggcagagagagcttctatagcacaggcagccagctgacccctgaccgatgtggacttcgttttgaggaacacaggcatcctgggcttggggaactgggacagggcccagacagctacggcagccccagtttccgcagcacaccggaggcaccctatgcctccctgacagagatagagcacctggtgcagagcgtctgcaagtcctacagggagacatgccagctgcggctggaggacctgctgcggcagcgctccaacatcttctcccgggaggaagtgactggctaccagaggaagtccatgtgggagatgtgggaacggtgtgcccaccacctcaccgaggccattcagtacgtggtggagttcgccaagaggctctcaggctttatggagctctgccagaatgaccagattgtgcttctcaaagcaggagcaatggaagtggtgctggttaggatgtgccgggcctacaatgctgacaaccgcacggtcttttttgaaggcaaatacggtggcatggagctgttccgagccttgggctgcagcgagctcatcagctccatctttgacttctcccactccctaagtgccttgcacttttccgaggatgagattgccctctacacagcccttgttctcatcaatgcccatcggccagggctccaagagaaaaggaaagtagaacagctgcagtacaatctggagctggcctttcatcatcatctctgcaagactcatcgccaaagcatcctggcaaagctgccacccaaggggaagcttcggagcctgtgtagccagcatgtggaaaggctgcagatcttccagcacctccaccccatcgtggtccaagccgctttccctccactctacaaggagctcttcagcactgaaaccgagtcacctgtggggctgtccaagtga

SEQ ID NO: 4 - DNA, 1488 bp, Mus musculus
atgagaacacaaattgaagtgatcccttgcaagatctgtggggacaagtcatctgggatccactacggggttatcacctgtgaggggtgcaagggcttcttccgccgcagccagcagtgtaatgtggcctactcctgcacgcgtcagcagaactgccccattgaccgaaccagccgcaaccgatgccagcattgccgcctgcagaagtgcctggctctgggcatgtcccgagatgctgtcaagtttggccgaatgtccaagaagcagagggacagtctacatgcagaagtgcagaaacaactgcaacagcagcagcaacaggaacaagtggccaagactcctccagctgggagccgcggagcagacacacttacatacactttagggctctcagatgggcagctaccactgggcgcctcacctgacctacccgaggcctctgcttgtccccctggcctcctgagagcctcaggctctggcccaccatattccaataccttggccaaaacagaggtccagggggcctcctgccaccttgagtatagtccagaacgaggcaaagctgaaggcagagacagcatctatagcactgacggccaacttactcttggaagatgtggacttcgttttgaggaaaccaggcatcctgaacttggggaaccagaacagggtccagacagccactgcattcccagtttctgcagtgccccagaggtaccatatgcctctctgacagacatagagtacctggtacagaatgtctgcaagtccttccgagagacatgccagctgcgactggaggaccttctacggcagcgcaccaacctcttttcacgggaggaggtgaccagctaccagaggaagtcaatgtgggagatgtgggagcgctgtgcccaccacctcactgaggccattcagtatgtggtggagtttgccaagcggctttcaggcttcatggagctctgccagaatgaccagatcatactactgaaagcaggagcaatggaagtcgtcctagtcagaatgtgcagggcctacaatgccaacaaccacacagtcttttttgaaggcaaatacggtggtgtggagctgtttcgagccttgggctgcagcgagctcatcagctccatatttgacttttcccacttcctcagcgccctgtgtttttctgaggatgagattgccctctacacggccctggttctcatcaatgccaaccgtcctgggctccaagagaagaggagagtggaacatctgcaatacaatttggaactggctttccatcatcatctctgcaagactcatcgacaaggcctcctagccaagctgccacccaaaggaaaactccggagcctgtgcagccaacatgtggaaaagctgcagatcttccagcacctccaccccatcgtggtccaagccgccttccctccactctataaggaactcttcagcactgatgttgaatcccctgaggggctgtcaaagtga

SEQ ID NO: 5 - protein, 497 aa, Homo sapiens
MRTQIEVIPCKICGDKSSGIHYGVITCEGCKGFFRRSQRCNAAYSCTRQQNCPIDRTSRNRCQHCRLQKCLALGMSRDAVKFGRMSKKQRDSLHAEVQKQLQQRQQQQQEPVVKTPPAGAQGADTLTYTLGLPDGQLPLGSSPDLPEASACPPGLLKASGSGPSYSNNLAKAGLNGASCHLEYSPERGKAEGRESFYSTGSQLTPDRCGLRFEEHRHPGLGELGQGPDSYGSPSFRSTPEAPYASLTEIEHLVQSVCKSYRETCQLRLEDLLRQRSNIFSREEVTGYQRKSMWEMWERCAHHLTEAIQYVVEFAKRLSGFMELCQNDQIVLLKAGAMEVVLVRMCRAYNADNRTVFFEGKYGGMELFRALGCSELISSIFDFSHSLSALHFSEDEIALYTALVLINAHRPGLQEKRKVEQLQYNLELAFHHHLCKTHRQSILAKLPPKGKLRSLCSQHVERLQIFQHLHPIVVQAAFPPLYKELFSTETESPVGLSK

SEQ ID NO: 6 - protein, 495 aa, Mus musculus
MRTQIEVIPCKICGDKSSGIHYGVITCEGCKGFFRRSQQCNVAYSCTRQQNCPIDRTSRNRCQHCRLQKCLALGMSRDAVKFGRMSKKQRDSLHAEVQKQLQQQQQQEQVAKTPPAGSRGADTLTYTLGLSDGQLPLGASPDLPEASACPPGLLRASGSGPPYSNTLAKTEVQGASCHLEYSPERGKAEGRDSIYSTDGQLTLGRCGLRFEETRHPELGEPEQGPDSHCIPSFCSAPEVPYASLTDIEYLVQNVCKSFRETCQLRLEDLLRQRTNLFSREEVTSYQRKSMWEMWERCAHHLTEAIQYVVEFAKRLSGFMELCQNDQIILLKAGAMEVVLVRMCRAYNANNHTVFFEGKYGGVELFRALGCSELISSIFDFSHFLSALCFSEDEIALYTALVLINANRPGLQEKRRVEHLQYNLELAFHHHLCKTHRQGLLAKLPPKGKLRSLCSQHVEKLQIFQHLHPIVVQAAFPPLYKELFSTDVESPEGLSK